European Patent Application EP 4 119 666 A1, published January 18, 2023. Title: Photoresponsive Protein for Color Recognition and Use Thereof. Applicant: Nagoya Institute of Technology. The sequence listing filed with the application follows.

SEQUENCE LISTING (6 sequences)

SEQ ID NO: 1 - protein, 367 aa, Guillardia thetaS
MTTSAPSLSDPNWQYGMGGWNNPRLPNFNLHDPTVIGVDWLGFLCLLGASLALMYKLMSFKGPDGDQEFFVGYREEKCLSIYVNLIAAITYWGRICAHFNNDMGLSLSVNYFKYLDYIFTCPILTLDLLWSLNLPYKITYSLFVGLTIACGVFCNAFEPPARYLWFMFGCFIFAFTWISIIRLVYARFQQFLNEDAKKIRAPLKLSLTLYFSIWCGYPALWLLTEFGAISQLAAHVMTVIMDVAAKSVYGFALLKFQLGVDKRDVWLDELKSVRYRDVVPQIRPSKTRESRMEYSEDGDFMRPSKGKRAEGDYMNPRWDHHDDGRRLPDSREMDEQVHEKDQEISSTMKQIADLNKQLSAMQESEAV

SEQ ID NO: 2 - DNA, 1101 bp, Guillardia theta
atgacgacgtctgccccttcactctccgatcccaactggcaatatggcatgggaggatggaacaatcctcgccttccaaacttcaatcttcacgacccgaccgtgatcggagttgattggctgggatttctttgtcttcttggtgcctctctcgccctcatgtacaagctcatgtcgttcaagggccccgatggcgaccaagagttcttcgtcggctaccgggaagagaagtgcctctccatctacgtcaacctcatcgctgccatcacctactggggccgtatctgcgctcacttcaacaatgacatgggcctttctctgtctgtcaactacttcaagtacctggactacatcttcacctgtcctatcctgacgctggatctgctgtggtcgctcaacctcccctacaagatcacctactctctcttcgtcggattgaccatcgcatgcggagtcttctgcaacgcgttcgagcctcccgcgcggtacctctggttcatgttcggctgcttcatctttgccttcacgtggatcagcatcatccgcctcgtctacgcgcggttccagcagtttctcaacgaggacgcgaagaagatccgagcgcctctcaagctctccctcaccctctacttcagcatctggtgcggctacccggccctctggcttctcaccgagttcggagccatctcccagctggcagcccacgtgatgactgtcatcatggacgtcgccgccaagtctgtgtacggcttcgccctgctcaagttccagctgggggtggacaagcgagacgtctggctcgatgagctcaagagcgtcaggtatcgtgacgtcgtccctcagatccgaccgtcgaagacgcgagagagccgcatggagtattcagaggacggagatttcatgcgtccgagcaaggggaagagggcggaaggagactacatgaaccctcgctgggaccaccatgacgatgggaggaggctgcccgacagccgggagatggacgagcaagtgcacgagaaggaccaggagatctcgtcgacgatgaagcagatcgccgacctcaacaagcagctctctgccatgcaggagtccgaggccgtt

SEQ ID NO: 3 - DNA, 36 bp, Artificial sequence
  Priemer
cgagctcaagcttatgatgacaacaagcgcccctag

SEQ ID NO: 4 - DNA, 35 bp, Artificial sequence
  Priemer
gaccggtggatcctgaacagcctcagactcttgca

SEQ ID NO: 5 - DNA, 21 bp, Artificial sequence
  Priemer
cataagcttgagctcgagatc

SEQ ID NO: 6 - DNA, 21 bp, Artificial sequence
  Priemer
caggatccaccggtcgccacc